European Patent Application EP 4 620 965 A1, published September 24, 2025. Title: Peptide having activities of skin condition improvement and uses thereof. Applicant: CAREGEN Co., LTD. The sequence listing filed with the application follows.

SEQUENCE LISTING (13 sequences)

SEQ ID NO: 1 - protein, 5 aa, synthetic construct
EVVDI

SEQ ID NO: 2 - DNA, 20 bp, synthetic construct
  source 1..20: mol_type = other DNA
caccctcaagagcctgagtc

SEQ ID NO: 3 - DNA, 20 bp, synthetic construct
  source 1..20: mol_type = other DNA
agacggctgagtagggaaca

SEQ ID NO: 4 - DNA, 20 bp, synthetic construct
  source 1..20: mol_type = other DNA
ccaggaaccgagtacaccat

SEQ ID NO: 5 - DNA, 20 bp, synthetic construct
  source 1..20: mol_type = other DNA
atacccaggttgggtgatga

SEQ ID NO: 6 - DNA, 20 bp, synthetic construct
  source 1..20: mol_type = other DNA
gcaagacctggctttggact

SEQ ID NO: 7 - DNA, 21 bp, synthetic construct
  source 1..21: mol_type = other DNA
gggagtttctggttagggctg

SEQ ID NO: 8 - DNA, 20 bp, synthetic construct
  source 1..20: mol_type = other DNA
ggagccaaaagggtcatcat

SEQ ID NO: 9 - DNA, 20 bp, synthetic construct
  source 1..20: mol_type = other DNA
gtgatggcatggactgtggt

SEQ ID NO: 10 - DNA, 20 bp, synthetic construct
  source 1..20: mol_type = other DNA
tcagtggctggaacagtgag

SEQ ID NO: 11 - DNA, 20 bp, synthetic construct
  source 1..20: mol_type = other DNA
tctggcatgtcccactatca

SEQ ID NO: 12 - DNA, 20 bp, synthetic construct
  source 1..20: mol_type = other DNA
ccttcttgggtgctggaata

SEQ ID NO: 13 - DNA, 20 bp, synthetic construct
  source 1..20: mol_type = other DNA
acacgataagggaggctgtg